European Patent Application EP 4 656 732 A1, published December 3, 2025. Title: 一种用于插入非天然氨基酸的体外无细胞蛋白质合成体系、方法及应用. Applicant: 康码（上海）生物科技有限公司. The sequence listing filed with the application follows.

SEQUENCE LISTING (21 sequences)

SEQ ID NO: 1 - DNA, 965 bp, synthetic construct
  source 1..965: mol_type = other DNA
atgatcaccgaaacctcttctccattcagatctatcttctctcactctggtaagcaccaccaccaccaccaccaccacggttagggtggggactacaaggatcacgacggggattacaaagaccatgatatcgattacaaggatgacgacgataagggatccagccatggaggaagcttggtttcttagggtgaagaattgttcaccggtgttgttccaatcttggttgaattggacggtgacgttaacggtcacaagttctctgttagaggtgaaggtgaaggtgacgctaccaacggtaagttgaccttgaagttcatctgtaccaccggtaagttgccagttccatggccaaccttggttaccaccttgacctacggtgttcaatgtttctctagatacccagaccacatgaagcaacacgacttcttcaagtctgctatgccagaaggttacgttcaagaaagaaccatctctttcaaggacgacggtacctacaagaccagagctgaagttaagttcgaaggtgacaccttggttaacagaatcgaattgaagggtatcgacttcaaggaagacggtaacatcttgggtcacaagttggaatacaacttcaactctcacaacgtttagatcaccgctgacaagcaaaagaacggtatcaaggctaacttcaagatcagacacaacgttgaagacggttctgttcaattggctgaccactaccaacaaaacaccccaatcggtgacggtccagttttgttgccagacaaccactacttgtctacccaatctaagttgtctaaggacccaaacgaaaagagagaccacatggttttgttggaattcgttaccgctgctggtatcaccttgggtatggacgaattgtacaagtaataaggattattacttggatgccaataaaaaaaaaaagcgacatagccgaactcgacgatcgctgctaa

SEQ ID NO: 2 - DNA, 71 bp, synthetic construct
  source 1..71: mol_type = other DNA
gggggacggtccggcgaccagcgggtctctaaaacctagccagcggggttcgacaccccggtctctcgcca

SEQ ID NO: 3 - DNA, 42 bp, synthetic construct
  source 1..42: mol_type = other DNA
accaccaccacggttagggtggggactacaaggatcacgacg

SEQ ID NO: 4 - DNA, 41 bp, synthetic construct
  source 1..41: mol_type = other DNA
ctccatggctggatcccttatcgtcgtcatccttgtaatcg

SEQ ID NO: 5 - DNA, 35 bp, synthetic construct
  source 1..35: mol_type = other DNA
ttgtagtccccaccctaaccgtggtggtggtggtg

SEQ ID NO: 6 - DNA, 41 bp, synthetic construct
  source 1..41: mol_type = other DNA
tacaaggatgacgacgataagggatccagccatggaggaag

SEQ ID NO: 7 - DNA, 45 bp, synthetic construct
  source 1..45: mol_type = other DNA
actctggtaagaaggaaaccgctgctgctaaattcgaacgccagc

SEQ ID NO: 8 - DNA, 46 bp, synthetic construct
  source 1..46: mol_type = other DNA
ccccaccctaaccgctgtccatgtgctggcgttcgaatttagcagc

SEQ ID NO: 9 - DNA, 46 bp, synthetic construct
  source 1..46: mol_type = other DNA
cagcggtttccttcttaccagagtgagagaagatagatctgaatgg

SEQ ID NO: 10 - DNA, 45 bp, synthetic construct
  source 1..45: mol_type = other DNA
cgccagcacatggacagcggttagggtggggactacaaggatcac

SEQ ID NO: 11 - DNA, 918 bp, synthetic construct
  source 1..918: mol_type = other DNA
atgatcaccgaaacctcttctccattcagatctatcttctctcactctggtaagaaggaaaccgctgctgctaaattcgaacgccagcacatggacagcggttagggtggggactacaaggatcacgacggggattacaaagaccatgatatcgattacaaggatgacgacgataagggatccagccatggaggaagcttggtttctaagggtgaagaattgttcaccggtgttgttccaatcttggttgaattggacggtgacgttaacggtcacaagttctctgttagaggtgaaggtgaaggtgacgctaccaacggtaagttgaccttgaagttcatctgtaccaccggtaagttgccagttccatggccaaccttggttaccaccttgacctacggtgttcaatgtttctctagatacccagaccacatgaagcaacacgacttcttcaagtctgctatgccagaaggttacgttcaagaaagaaccatctctttcaaggacgacggtacctacaagaccagagctgaagttaagttcgaaggtgacaccttggttaacagaatcgaattgaagggtatcgacttcaaggaagacggtaacatcttgggtcacaagttggaatacaacttcaactctcacaacgtttacatcaccgctgacaagcaaaagaacggtatcaaggctaacttcaagatcagacacaacgttgaagacggttctgttcaattggctgaccactaccaacaaaacaccccaatcggtgacggtccagttttgttgccagacaaccactacttgtctacccaatctaagttgtctaaggacccaaacgaaaagagagaccacatggttttgttggaattcgttaccgctgctggtatcaccttgggtatggacgaattgtacaagtaa

SEQ ID NO: 12 - DNA, 42 bp, synthetic construct
  source 1..42: mol_type = other DNA
accaccaccaccacggttagggtggggactacaaggatcacg

SEQ ID NO: 13 - DNA, 41 bp, synthetic construct
  source 1..41: mol_type = other DNA
tccttgtagtccccaccctaaccgtggtggtggtggtggtg

SEQ ID NO: 14 - DNA, 43 bp, synthetic construct
  source 1..43: mol_type = other DNA
aactctcacaacgtttagatcaccgctgacaagcaaaagaacg

SEQ ID NO: 15 - DNA, 44 bp, synthetic construct
  source 1..44: mol_type = other DNA
tgtcagcggtgatctaaacgttgtgagagttgaagttgtattcc

SEQ ID NO: 16 - DNA, 5914 bp, synthetic construct
  source 1..5914: mol_type = other DNA
tggcgaatgggacgcgccctgtagcggcgcattaagcgcggcgggtgtggtggttacgcgcagcgtgaccgctacacttgccagcgccctagcgcccgctcctttcgctttcttcccttcctttctcgccacgttcgccggctttccccgtcaagctctaaatcgggggctccctttagggttccgatttagtgctttacggcacctcgaccccaaaaaacttgattagggtgatggttcacgtagtgggccatcgccctgatagacggtttttcgccctttgacgttggagtccacgttctttaatagtggactcttgttccaaactggaacaacactcaaccctatctcggtctattcttttgatttataagggattttgccgatttcggcctattggttaaaaaatgagctgatttaacaaaaatttaacgcgaattttaacaaaatattaacgtttacaatttcaggtggcacttttcggggaaatgtgcgcggaacccctatttgtttatttttctaaatacattcaaatatgtatccgctcatgagacaataaccctgataaatgcttcaataatattgaaaaaggaagagtatgagtattcaacatttccgtgtcgcccttattcccttttttgcggcattttgccttcctgtttttgctcacccagaaacgctggtgaaagtaaaagatgctgaagatcagttgggtgcacgagtgggttacatcgaactggatctcaacagcggtaagatccttgagagttttcgccccgaagaacgttttccaatgatgagcacttttaaagttctgctatgtggcgcggtattatcccgtattgacgccgggcaagagcaactcggtcgccgcatacactattctcagaatgacttggttgagtactcaccagtcacagaaaagcatcttacggatggcatgacagtaagagaattatgcagtgctgccataaccatgagtgataacactgcggccaacttacttctgacaacgatcggaggaccgaaggagctaaccgcttttttgcacaacatgggggatcatgtaactcgccttgatcgttgggaaccggagctgaatgaagccataccaaacgacgagcgtgacaccacgatgcctgcagcaatggcaacaacgttgcgcaaactattaactggcgaactacttactctagcttcccggcaacaattaatagactggatggaggcggataaagttgcaggaccacttctgcgctcggcccttccggctggctggtttattgctgataaatctggagccggtgagcgtgggtctcgcggtatcattgcagcactggggccagatggtaagccctcccgtatcgtagttatctacacgacggggagtcaggcaactatggatgaacgaaatagacagatcgctgagataggtgcctcactgattaagcattggtaactgtcagaccaagtttactcatatatactttagattgatttaaaacttcatttttaatttaaaaggatctaggtgaagatcctttttgataatctcatgaccaaaatcccttaacgtgagttttcgttccactgagcgtcagaccccgtagaaaagatcaaaggatcttcttgagatcctttttttctgcgcgtaatctgctgcttgcaaacaaaaaaaccaccgctaccagcggtggtttgtttgccggatcaagagctaccaactctttttccgaaggtaactggcttcagcagagcgcagataccaaatactgttcttctagtgtagccgtagttaggccaccacttcaagaactctgtagcaccgcctacatacctcgctctgctaatcctgttaccagtggctgctgccagtggcgataagtcgtgtcttaccgggttggactcaagacgatagttaccggataaggcgcagcggtcgggctgaacggggggttcgtgcacacagcccagcttggagcgaacgacctacaccgaactgagatacctacagcgtgagctatgagaaagcgccacgcttcccgaagggagaaaggcggacaggtatccggtaagcggcagggtcggaacaggagagcgcacgagggagcttccagggggaaacgcctggtatctttatagtcctgtcgggtttcgccacctctgacttgagcgtcgatttttgtgatgctcgtcaggggggcggagcctatggaaaaacgccagcaacgcggcctttttacggttcctggccttttgctggccttttgctcacatgttctttcctgcgttatcccctgattctgtggataaccgtattaccgcctttgagtgagctgataccgctcgccgcagccgaacgaccgagcgcagcgagtcagtgagcgaggaagcggaagagcgcccaatacgcaaaccgcctctccccgcgcgttggccgattcattaatgcagctggcacgacaggtttcccgactggaaagcgggcagtgagcgcaacgcaattgatgcctccgtgtaagggggatttctgttcatgggggtaatgataccgatgaaacgagagaggatgctcacgatacgggttactgatgatgaacatgcccggttactggaacgttgtgagggtaaacaactggcggtatggatgcggcgggaccagagaaaaatcactcagggtcaatgccagcgcttcgttaatacagatgtaggtgttccacagggtagccagcagcatcctgcgatgcagatccggaacataatggtgcagggcgctgacttccgcgtttccagactttacgaaacacggaaaccgaagaccattcatgttgttgctcaggtcgcagacgttttgcagcagcagtcgcttcacgttcgctcgcgtatcggtgattcattctgctaaccagtaaggcaaccccgccagcctagccgggtcctcaacgacaggagcacgatcatgcgcacccgtggggccgccatgccggcgataatggcctgcttctcgccgaaacgtttggtggcgggaccagtgacgaaggcttgagcgagggcgtgcaagattccgaataccgcaagcgacaggccgatcatcgtcgcgctccagcgaaagcggtcctcgccgaaaatgacccagagcgctgccggcacctgtcctacgagttgcatgataaagaagacagtcataagtgcggcgacgatagtcatgccccgcgcccaccggaaggagctgactgggttgaaggctctcaagggcatcggtcgagatcccggtgcctaatgagtgagctaacttacattaattgcgttgcgctcactgcccgctttccagtcgggaaacctgtcgtgccagctgcattaatgaatcggccaacgcgcggggagaggcggtttgcgtattgggcgccagggtggtttttcttttcaccagtgagacgggcaacagctgattgcccttcaccgcctggccctgagagagttgcagcaagcggtccacgctggtttgccccagcaggcgaaaatcctgtttgatggtggttaacggcgggatataacatgagctgtcttcggtatcgtcgtatcccactaccgagatatccgcaccaacgcgcagcccggactcggtaatggcgcgcattgcgcccagcgccatctgatcgttggcaaccagcatcgcagtgggaacgatgccctcattcagcatttgcatggtttgttgaaaaccggacatggcactccagtcgccttcccgttccgctatcggctgaatttgattgcgagtgagatatttatgccagccagccagacgcagacgcgccgagacagaacttaatgggcccgctaacagcgcgatttgctggtgacccaatgcgaccagatgctccacgcccagtcgcgtaccgtcttcatgggagaaaataatactgttgatgggtgtctggtcagagacatcaagaaataacgccggaacattagtgcaggcagcttccacagcaatggcatcctggtcatccagcggatagttaatgatcagcccactgacgcgttgcgcgagaagattgtgcaccgccgctttacaggcttcgacgccgcttcgttctaccatcgacaccaccacgctggcacccagttgatcggcgcgagatttaatcgccgcgacaatttgcgacggcgcgtgcagggccagactggaggtggcaacgccaatcagcaacgactgtttgcccgccagttgttgtgccacgcggttgggaatgtaattcagctccgccatcgccgcttccactttttcccgcgttttcgcagaaacgtggctggcctggttcaccacgcgggaaacggtctgataagagacaccggcatactctgcgacatcgtataacgttactggtttcacattcaccaccctgaattgactctcttccgggcgctatcatgccataccgcgaaaggttttgcgccattcgatggtgtccgggatctcgacgctctcccttatgcgactcctgcattaggaagcagcccagtagtaggttgaggccgttgagcaccgccgccgcaaggaatggtgcatgcaaggagatggcgcccaacagtcccccggccacggggcctgccaccatacccacgccgaaacaagcgctcatgagcccgaagtggcgagcccgatcttccccatcggtgatgtcggcgatataggcgccagcaaccgcacctgtggcgccggtgatgccggccacgatgcgtccggcgtagaggatcgagatctcgcgaaattaatacgactcactatagggaaaaaagaaatctctcaagctgaaattaaaccaaaactctaatataagaaaaaaaaatagaaaggtatttttacaacaattaccaacaacaacaaacaacaaacaacattacaattactatttacaattacaaaaaaaaaaaatgatcaccgaaacctcttctccattcagatctatcttctctcactctggtaagcaccaccaccaccaccaccaccacggttctggtggatccagccatggaggaagcttggtttctaagggtgaagaattgttcaccggtgttgttccaatcttggttgaattggacggtgacgttaacggtcacaagttctctgttagaggtgaaggtgaaggtgacgctaccaacggtaagttgaccttgaagttcatctgtaccaccggtaagttgccagttccatggccaaccttggttaccaccttgacctacggtgttcaatgtttctctagatacccagaccacatgaagcaacacgacttcttcaagtctgctatgccagaaggttacgttcaagaaagaaccatctctttcaaggacgacggtacctacaagaccagagctgaagttaagttcgaaggtgacaccttggttaacagaatcgaattgaagggtatcgacttcaaggaagacggtaacatcttgggtcacaagttggaatacaacttcaactctcacaacgtttacatcaccgctgacaagcaaaagaacggtatcaaggctaacttcaagatcagacacaacgttgaagacggttctgttcaattggctgaccactaccaacaaaacaccccaatcggtgacggtccagttttgttgccagacaaccactacttgtctacccaatctaagttgtctaaggacccaaacgaaaagagagaccacatggttttgttggaattcgttaccgctgctggtatcaccttgggtatggacgaattgtacaagtaaataaggattaattacttggatgccaataaaaaaaaaaaagcgacatagcccgaactcgacgatccggctgctaacaaagcccgaaaggaagctgagttggctgctgccaccgctgagcaataactgaaaggaggaactatatccggat

SEQ ID NO: 17 - DNA, 802 bp, synthetic construct
  source 1..802: mol_type = other DNA
atgatcaccgaaacctcttctccattcagatctatcttctctcactctggtaagcaccaccaccaccaccaccaccacggttagggtggggactacaaggatcacgacggggattacaaagaccatgatatcgattacaaggatgacgacgataagggatccagccatggaggaagcttggtttctaagggtgaagaattgttcaccggtgttgttccaatcttggttgaattggacggtgacgttaacggtcacaagttctctgttagaggtgaaggtgaaggtgacgctaccaacggtaagttgaccttgaagttcatctgtaccaccggtaagttgccagttccatggccaaccttggttaccaccttgacctacggtgttcaatgtttctctagatacccagaccacatgaagcaacacgacttcttcaagtctgctatgccagaaggttacgttcaagaaagaaccatctctttcaaggacgacggtacctacaagaccagagctgaagttaagttcgaaggtgacaccttggttaacagaatcgaattgaagggtatcgacttcaaggaagacggtaacatcttgggtcacaagttggaatacaacttcaactctcacaacgtttagatcaccgctgacaagcaaaagaacggtatcaaggctaacttcaagatcagacacaacgttgaagacggttctgttcaattggctgaccactaccaacaaaacaccccaatcggtgacggtccagttttgttgccagacaaccactacttgtctacccaatctaagttgt

SEQ ID NO: 18 - DNA, 24 bp, synthetic construct
  source 1..24: mol_type = other DNA
ggtgatgtcggcgatataggcgcc

SEQ ID NO: 19 - DNA, 24 bp, synthetic construct
  source 1..24: mol_type = other DNA
tgctcagcggtggcagcagccaac

SEQ ID NO: 20 - DNA, 44 bp, synthetic construct
  source 1..44: mol_type = other DNA
caaggacgacggttagtacaagaccagagctgaagttaagttcg

SEQ ID NO: 21 - DNA, 41 bp, synthetic construct
  source 1..41: mol_type = other DNA
cagctctggtcttgtactaaccgtcgtccttgaaagagatg